European Patent Application EP 4 592 305 A2, published July 30, 2025. Title: PRODUCTION OF CYCLIC ADENYLATES AND THEIR USE AS ALLOSTERIC REGULATORS. Applicant: Vilnius University. Application EP. The sequence listing filed with the application follows.

SEQUENCE LISTING (26 sequences)

SEQ ID NO: 1 - protein, 4 aa, Streptococcus thermophilus
GGDD

SEQ ID NO: 2 - protein, 10 aa, Streptococcus thermophilus
  SITE 3: note = misc_feature - Xaa can be any naturally occurring amino acid
  REGION 6..8: note = misc_feature - Xaa can be any naturally occurring amino acid
DNXSTXXXRK

SEQ ID NO: 3 - protein, 190 aa, Streptococcus thermophilus
VEDLDALWERYREAVRAGGNPQALYQEMVWPALLALWREKPRVYPFPQAFAVSVHTLGTSPEATALAILGAGAERVYVLHTPESARFLPRLRQDTGKDLYPVEIGKSDVEAIYREVKRLLEKHPEVPVALDLTSGTKAMSAGLAAAGFFFQRFYPKVRVVYVDNEDYDPELRRPRAGTEKLRILPNPHEA

SEQ ID NO: 4 - protein, 180 aa, Streptococcus thermophilus
MKILFSPIGNSDPWRNDRDGAMLHIVRHYNLDKVVLYFTRTIWEGNENRKGHKIYEWEKIIQTVSPNTEVEIIIENVDNAQDYDVFKEKFHKYLKIIEDSYEDCEIILNVTSGTPQMESTLCLEYIVYPENKKCVQVSTPTKDSNAGIEYSNPKDKVEEFEIVNEVEKKSEKRCKEINIL

SEQ ID NO: 5 - protein, 173 aa, Streptococcus thermophilus
LKILISAVGTTDPISNNHDAALLHIARNYRPDKIVLVYSQEMMVKQDLINKVLLSIEGYNPIIEIDSTILNNDEVFLFDKMYEVMGQIVQKYTNDDNEIILNLSSGTPQIISALFALNRINDYNTQAIQVATPKNRANREYTALTESEIDALIMENQDNRLDFVDRSIKDKSE

SEQ ID NO: 6 - protein, 174 aa, Streptococcus thermophilus
MRVLISAVGDTDPFRNFHDGSLIHIARKYRPEKVILIFSEHTAKKQGNIEKALFSIAPNYEPELIIHDPIISDNEVHIFDVMFQRFSDILQEYYTKEDEFILNLSSATPQIKSALFVINRLNGINVKAVQVSSPEHASNENIGHDNDENIDELIEVNKDNKVNFIDRTIEDNAE

SEQ ID NO: 7 - protein, 254 aa, Streptococcus thermophilus
TEQETLTILLDVYAYYQAYQIVKASQFFSDDIIFLLELLKERRELNVDFLFQNQVHLQELELTYHISLLDNAYEEELLANYIMDLEAKLRNDHIIDFVRSVSPILYRLLMRLMQSQVADINDYIYDAKNDQYDTWKFDKMHDSANPFVQNFVAKGRDSKITSRSLADFIQLTDLPQAIKDNILLLRDFEKSVRNPLAHLIKPFDEEELHRTTGFSSQTFLEKIIQLAVFSGIHYDNDKFYFDKVNELIKRIYQN

SEQ ID NO: 8 - protein, 242 aa, Streptococcus thermophilus
SFREAMIRSQILGLIDNYDYEGALNLVSNQKSFRNGKLLRKKLLSLTKQIKTHEVFPEINEKYRDDALKKSLFHYLLLNMRYNRLDVAETLIRVKSIAEFILKTYIEIHWPTLIIEKDGKPYLNDEDNLSFVYKYNLLLEKRKQNFDVSRILGLPAFIDILTILEPNSQLLKEVNAVNDINGLRNSIAHNLDTLNLDKNKNYKKIMLSVEAIKNMLHISFPEIEEEDYNYFEEKNKEFKELL

SEQ ID NO: 9 - protein, 255 aa, Streptococcus thermophilus
KFTQALVKRHLRSLIASFDYQAAEAIINRKEYNKLLSKKKIAYIREKLYDFSRVFKNQSILSDILSFPLDDSQKKALNYYLMIDVLKEREHIADVLIKAKSLAEFVIEETIKKDHEGLIVFDGNLPKLNPSFPDCEAILDDIDKKMKKSRGIEDTEERIFSVQSTLNLLSYLNILEFYEYDSQLQTAINGILSLNGERNKVAHGLSEIDTRLLSRKKLKQLSENLRLLLVDCLGIDSSYFNYYDKQNKELIKMLE

SEQ ID NO: 10 - protein, 212 aa, Streptococcus thermophilus
KFSQALLKKTARDFIEKFDYKAALDILDQLSDFPNLKSVREEIRDVVNCLSKQDVPKGLRHKKLKEEEQKILSAYLTIELQRERGNVSESFIRIKNLTEFILEDYIEKRYPGLIDEYCEDIQKYYLSLFDYSKLLKATKEFKLKRTIAPIIDMNSSRNKVAHSLSPLDSDAVKQLGIAMKTLKTLVREQYHFSQSDFNFYHDLNKILLTKLN

SEQ ID NO: 11 - RNA, 68 nt, synthetic construct
  misc_feature 1..68: note = RNA NS
  source 1..68: mol_type = other RNA
gggcggcaaattgaggatttcgtaactgtttaattctgttcacttattccaccaacaaaaggtggcga

SEQ ID NO: 12 - RNA, 78 nt, synthetic construct
  misc_feature 1..78: note = RNA NSc
  source 1..78: mol_type = other RNA
gggaaacagcatagcaagttaaaataaggctagtccgttatcaacttgaaaaagtggcaccgagtcggtgcttttttt

SEQ ID NO: 13 - RNA, 80 nt, synthetic construct
  misc_feature 1..80: note = RNA NSd
  source 1..80: mol_type = other RNA
gggtaaatcttgcagaagctacaaagataaggcttcatgccgaaatcaacaccctgtcattttatggcagggtgttttcg

SEQ ID NO: 14 - skipped

SEQ ID NO: 15 - RNA, 52 nt, synthetic construct
  misc_feature 1..52: note = RNA NSe
  source 1..52: mol_type = other RNA
gggtttcccaaccatccagcctaccggccgtccgacctgccttccctttccc

SEQ ID NO: 16 - RNA, 40 nt, Streptococcus thermophilus
  source 1..40: mol_type = other RNA
cttattcacttgtcttaatttgtcaatgctttcaaaggca

SEQ ID NO: 17 - RNA, 68 nt, synthetic construct
  misc_feature 1..68: note = RNA S3/2
  source 1..68: mol_type = other RNA
gggatccccaaatataaggtggaataagtgaacagaattaaacagttacgaaaaaaaaaaagggtacc

SEQ ID NO: 18 - RNA, 68 nt, synthetic construct
  misc_feature 1..68: note = RNA S3/3
  source 1..68: mol_type = other RNA
gggatccccaaatataaggtggaataagtgaacagaattaaacagttacgaaagtttccgtgggtacc

SEQ ID NO: 19 - RNA, 68 nt, synthetic construct
  misc_feature 1..68: note = RNA S3/7
  source 1..68: mol_type = other RNA
gggatccccaaatataaggtggaataagtgaacagaattaaacagttacctaaaaaaaaaagggtacc

SEQ ID NO: 20 - RNA, 68 nt, synthetic construct
  misc_feature 1..68: note = RNA S3/15
  source 1..68: mol_type = other RNA
gggatccccaaatataaggtggataaagtgaacagaattaaacagttacgaaaaaaaaaaagggtacc

SEQ ID NO: 21 - RNA, 68 nt, synthetic construct
  misc_feature 1..68: note = RNA S3/9
  source 1..68: mol_type = other RNA
gggatccccaaatataaggtggaataagtgaacactattaaacagttacgaaaaaaaaaaagggtacc

SEQ ID NO: 22 - RNA, 53 nt, synthetic construct
  misc_feature 1..53: note = RNA S3/10
  source 1..53: mol_type = other RNA
gggatccccaaatataaggtggaataagtgaacagaattaaacagttacgaaa

SEQ ID NO: 23 - RNA, 48 nt, synthetic construct
  misc_feature 1..48: note = RNA S3/14
  source 1..48: mol_type = other RNA
ggaataagtgaacagaattaaacagttacgaaaaaaaaaaagggtacc

SEQ ID NO: 24 - RNA, 84 nt, synthetic construct
  misc_feature 1..84: note = ssRNA NSa
  source 1..84: mol_type = other RNA
gggtaccgagctcgaattgaaattctaaacgctaaagaggaagaggacatggtgaattcgtaatcatggtcatagctgtttccc

SEQ ID NO: 25 - RNA, 84 nt, synthetic construct
  misc_feature 1..84: note = ssRNA NSb
  source 1..84: mol_type = other RNA
gggaaacagctatgaccatgattacgaattcaccatgtcctcttcctctttagcgtttagaatttcaattcgagctcggtaccc

SEQ ID NO: 26 - DNA, 52 bp, synthetic construct
  misc_feature 1..52: note = ssDNA S3/2
  source 1..52: mol_type = other DNA
aaatataaggtggaataagtgaacagaattaaacagttacgaaaaaaaaaaa